European Patent Application EP 4 707 392 A1, published March 11, 2026. Title: DOUBLE-STRANDED OLIGONUCLEOTIDE, CONJUGATE THEREOF, AND USE THEREOF. Applicant: RIGERNA THERAPEUTICS (BEIJING) CO., LTD. Application US. The sequence listing filed with the application follows.

SEQUENCE LISTING (614 sequences)

SEQ ID NO: 1 - RNA, 19 nt, synthetic construct
  source 1..19: mol_type = other RNA
cagacagacaagaccatct

SEQ ID NO: 2 - RNA, 21 nt, synthetic construct
  source 1..21: mol_type = other RNA
agatggtcttgtctgtctgga

SEQ ID NO: 3 - RNA, 19 nt, synthetic construct
  source 1..19: mol_type = other RNA
cagacagacaagaccatct

SEQ ID NO: 4 - RNA, 21 nt, synthetic construct
  source 1..21: mol_type = other RNA
agatggtcttgtctgtctgga

SEQ ID NO: 5 - RNA, 19 nt, synthetic construct
  source 1..19: mol_type = other RNA
cagacagacaagaccatct

SEQ ID NO: 6 - RNA, 21 nt, synthetic construct
  source 1..21: mol_type = other RNA
agatggtcttgtctgtctgga

SEQ ID NO: 7 - RNA, 19 nt, synthetic construct
  source 1..19: mol_type = other RNA
cagacagacaagaccatct

SEQ ID NO: 8 - RNA, 21 nt, synthetic construct
  source 1..21: mol_type = other RNA
agatggtcttgtctgtctgga

SEQ ID NO: 9 - RNA, 19 nt, synthetic construct
  source 1..19: mol_type = other RNA
cagacagacaagaccatct

SEQ ID NO: 10 - RNA, 21 nt, synthetic construct
  source 1..21: mol_type = other RNA
agatggtcttgtctgtctgga

SEQ ID NO: 11 - RNA, 19 nt, synthetic construct
  source 1..19: mol_type = other RNA
cagacagacaagaccatct

SEQ ID NO: 12 - RNA, 21 nt, synthetic construct
  source 1..21: mol_type = other RNA
agatggtcttgtctgtctgga

SEQ ID NO: 13 - RNA, 19 nt, synthetic construct
  source 1..19: mol_type = other RNA
cagacagacaagaccatct

SEQ ID NO: 14 - RNA, 21 nt, synthetic construct
  source 1..21: mol_type = other RNA
agatggtcttgtctgtctgga

SEQ ID NO: 15 - RNA, 19 nt, synthetic construct
  source 1..19: mol_type = other RNA
cagacagacaagaccatct

SEQ ID NO: 16 - RNA, 21 nt, synthetic construct
  source 1..21: mol_type = other RNA
agatggtcttgtctgtctgga

SEQ ID NO: 17 - RNA, 19 nt, synthetic construct
  source 1..19: mol_type = other RNA
cagacagacaagaccatct

SEQ ID NO: 18 - RNA, 21 nt, synthetic construct
  source 1..21: mol_type = other RNA
agatggtcttgtctgtctgga

SEQ ID NO: 19 - RNA, 19 nt, synthetic construct
  source 1..19: mol_type = other RNA
cagacagacaagaccatct

SEQ ID NO: 20 - RNA, 21 nt, synthetic construct
  source 1..21: mol_type = other RNA
agatggtcttgtctgtctgga

SEQ ID NO: 21 - RNA, 19 nt, synthetic construct
  source 1..19: mol_type = other RNA
cagacagacaagaccatct

SEQ ID NO: 22 - RNA, 21 nt, synthetic construct
  source 1..21: mol_type = other RNA
agatggtcttgtctgtctgga

SEQ ID NO: 23 - RNA, 19 nt, synthetic construct
  source 1..19: mol_type = other RNA
cagacagacaagaccatct

SEQ ID NO: 24 - RNA, 21 nt, synthetic construct
  source 1..21: mol_type = other RNA
agatggtcttgtctgtctgga

SEQ ID NO: 25 - RNA, 19 nt, synthetic construct
  source 1..19: mol_type = other RNA
cagacagacaagaccatct

SEQ ID NO: 26 - RNA, 21 nt, synthetic construct
  source 1..21: mol_type = other RNA
agatggtcttgtctgtctgga

SEQ ID NO: 27 - RNA, 19 nt, synthetic construct
  source 1..19: mol_type = other RNA
cagacagacaagaccatct

SEQ ID NO: 28 - RNA, 21 nt, synthetic construct
  source 1..21: mol_type = other RNA
agatggtcttgtctgtctgga

SEQ ID NO: 29 - RNA, 19 nt, synthetic construct
  source 1..19: mol_type = other RNA
cagacagacaagaccatct

SEQ ID NO: 30 - RNA, 21 nt, synthetic construct
  source 1..21: mol_type = other RNA
agatggtcttgtctgtctgga

SEQ ID NO: 31 - RNA, 19 nt, synthetic construct
  source 1..19: mol_type = other RNA
cagacagacaagaccatct

SEQ ID NO: 32 - RNA, 21 nt, synthetic construct
  source 1..21: mol_type = other RNA
agatggtcttgtctgtctgga

SEQ ID NO: 33 - RNA, 19 nt, synthetic construct
  source 1..19: mol_type = other RNA
cagacagacaagaccatct

SEQ ID NO: 34 - RNA, 21 nt, synthetic construct
  source 1..21: mol_type = other RNA
agatggtcttgtctgtctgga

SEQ ID NO: 35 - RNA, 19 nt, synthetic construct
  source 1..19: mol_type = other RNA
cagacagacaagaccatct

SEQ ID NO: 36 - RNA, 21 nt, synthetic construct
  source 1..21: mol_type = other RNA
agatggtcttgtctgtctgga

SEQ ID NO: 37 - RNA, 19 nt, synthetic construct
  source 1..19: mol_type = other RNA
cagacagacaagaccatct

SEQ ID NO: 38 - RNA, 21 nt, synthetic construct
  source 1..21: mol_type = other RNA
agatggtcttgtctgtctgga

SEQ ID NO: 39 - RNA, 19 nt, synthetic construct
  source 1..19: mol_type = other RNA
cagacagacaagaccatct

SEQ ID NO: 40 - RNA, 21 nt, synthetic construct
  source 1..21: mol_type = other RNA
agatggtcttgtctgtctgga

SEQ ID NO: 41 - RNA, 19 nt, synthetic construct
  source 1..19: mol_type = other RNA
cagacagacaagaccatct

SEQ ID NO: 42 - RNA, 21 nt, synthetic construct
  source 1..21: mol_type = other RNA
agatggtcttgtctgtctgga

SEQ ID NO: 43 - RNA, 19 nt, synthetic construct
  source 1..19: mol_type = other RNA
cagacagacaagaccatct

SEQ ID NO: 44 - RNA, 21 nt, synthetic construct
  source 1..21: mol_type = other RNA
agatggtcttgtctgtctgga

SEQ ID NO: 45 - RNA, 19 nt, synthetic construct
  source 1..19: mol_type = other RNA
cagacagacaagaccatct

SEQ ID NO: 46 - RNA, 21 nt, synthetic construct
  source 1..21: mol_type = other RNA
agatggtcttgtctgtctgga

SEQ ID NO: 47 - RNA, 19 nt, synthetic construct
  source 1..19: mol_type = other RNA
cagacagacaagaccatct

SEQ ID NO: 48 - RNA, 21 nt, synthetic construct
  source 1..21: mol_type = other RNA
agatggtcttgtctgtctgga

SEQ ID NO: 49 - RNA, 19 nt, synthetic construct
  source 1..19: mol_type = other RNA
cagacagacaagaccatct

SEQ ID NO: 50 - RNA, 21 nt, synthetic construct
  source 1..21: mol_type = other RNA
agatggtcttgtctgtctgga

SEQ ID NO: 51 - RNA, 19 nt, synthetic construct
  source 1..19: mol_type = other RNA
cagacagacaagaccatct

SEQ ID NO: 52 - RNA, 21 nt, synthetic construct
  source 1..21: mol_type = other RNA
agatggtcttgtctgtctgga

SEQ ID NO: 53 - RNA, 19 nt, synthetic construct
  source 1..19: mol_type = other RNA
cagacagacaagaccatct

SEQ ID NO: 54 - RNA, 21 nt, synthetic construct
  source 1..21: mol_type = other RNA
agatggtcttgtctgtctgga

SEQ ID NO: 55 - RNA, 19 nt, synthetic construct
  source 1..19: mol_type = other RNA
cagacagacaagaccatct

SEQ ID NO: 56 - RNA, 21 nt, synthetic construct
  source 1..21: mol_type = other RNA
agatggtcttgtctgtctgga

SEQ ID NO: 57 - RNA, 19 nt, synthetic construct
  source 1..19: mol_type = other RNA
cagacagacaagaccatct

SEQ ID NO: 58 - RNA, 21 nt, synthetic construct
  source 1..21: mol_type = other RNA
agatggtcttgtctgtctgga

SEQ ID NO: 59 - RNA, 19 nt, synthetic construct
  source 1..19: mol_type = other RNA
cagacagacaagaccatct

SEQ ID NO: 60 - RNA, 21 nt, synthetic construct
  source 1..21: mol_type = other RNA
agatggtcttgtctgtctgga

SEQ ID NO: 61 - RNA, 19 nt, synthetic construct
  source 1..19: mol_type = other RNA
cagacagacaagaccatct

SEQ ID NO: 62 - RNA, 21 nt, synthetic construct
  source 1..21: mol_type = other RNA
agatggtcttgtctgtctgga

SEQ ID NO: 63 - RNA, 19 nt, synthetic construct
  source 1..19: mol_type = other RNA
cagacagacaagaccatct

SEQ ID NO: 64 - RNA, 21 nt, synthetic construct
  source 1..21: mol_type = other RNA
agatggtcttgtctgtctgga

SEQ ID NO: 65 - RNA, 19 nt, synthetic construct
  source 1..19: mol_type = other RNA
cagacagacaagaccatct

SEQ ID NO: 66 - RNA, 21 nt, synthetic construct
  source 1..21: mol_type = other RNA
agatggtcttgtctgtctgga

SEQ ID NO: 67 - RNA, 19 nt, synthetic construct
  source 1..19: mol_type = other RNA
cagacagacaagaccatct

SEQ ID NO: 68 - RNA, 21 nt, synthetic construct
  source 1..21: mol_type = other RNA
agatggtcttgtctgtctgga

SEQ ID NO: 69 - RNA, 19 nt, synthetic construct
  source 1..19: mol_type = other RNA
cagacagacaagaccatct

SEQ ID NO: 70 - RNA, 21 nt, synthetic construct
  source 1..21: mol_type = other RNA
agatggtcttgtctgtctgga

SEQ ID NO: 71 - RNA, 19 nt, synthetic construct
  source 1..19: mol_type = other RNA
cagacagacaagaccatct

SEQ ID NO: 72 - RNA, 21 nt, synthetic construct
  source 1..21: mol_type = other RNA
agatggtcttgtctgtctgga

SEQ ID NO: 73 - RNA, 19 nt, synthetic construct
  source 1..19: mol_type = other RNA
cagacagacaagaccatct

SEQ ID NO: 74 - RNA, 21 nt, synthetic construct
  source 1..21: mol_type = other RNA
agatggtcttgtctgtctgga

SEQ ID NO: 75 - RNA, 19 nt, synthetic construct
  source 1..19: mol_type = other RNA
cagacagacaagaccatct

SEQ ID NO: 76 - RNA, 21 nt, synthetic construct
  source 1..21: mol_type = other RNA
agatggtcttgtctgtctgga

SEQ ID NO: 77 - RNA, 19 nt, synthetic construct
  source 1..19: mol_type = other RNA
cagacagacaagaccatct

SEQ ID NO: 78 - RNA, 21 nt, synthetic construct
  source 1..21: mol_type = other RNA
agatggtcttgtctgtctgga

SEQ ID NO: 79 - RNA, 19 nt, synthetic construct
  source 1..19: mol_type = other RNA
cagacagacaagaccatct

SEQ ID NO: 80 - RNA, 21 nt, synthetic construct
  source 1..21: mol_type = other RNA
agatggtcttgtctgtctgga

SEQ ID NO: 81 - RNA, 19 nt, synthetic construct
  source 1..19: mol_type = other RNA
cagacagacaagaccatct

SEQ ID NO: 82 - RNA, 21 nt, synthetic construct
  source 1..21: mol_type = other RNA
agatggtcttgtctgtctgga

SEQ ID NO: 83 - RNA, 19 nt, synthetic construct
  source 1..19: mol_type = other RNA
cagacagacaagaccatct

SEQ ID NO: 84 - RNA, 21 nt, synthetic construct
  source 1..21: mol_type = other RNA
agatggtcttgtctgtctgga

SEQ ID NO: 85 - RNA, 19 nt, synthetic construct
  source 1..19: mol_type = other RNA
cagacagacaagaccatct

SEQ ID NO: 86 - RNA, 21 nt, synthetic construct
  source 1..21: mol_type = other RNA
agatggtcttgtctgtctgga

SEQ ID NO: 87 - RNA, 19 nt, synthetic construct
  source 1..19: mol_type = other RNA
cagacagacaagaccatct

SEQ ID NO: 88 - RNA, 21 nt, synthetic construct
  source 1..21: mol_type = other RNA
agatggtcttgtctgtctgga

SEQ ID NO: 89 - RNA, 19 nt, synthetic construct
  source 1..19: mol_type = other RNA
cagacagacaagaccatct

SEQ ID NO: 90 - RNA, 21 nt, synthetic construct
  source 1..21: mol_type = other RNA
agatggtcttgtctgtctgga

SEQ ID NO: 91 - RNA, 19 nt, synthetic construct
  source 1..19: mol_type = other RNA
cagacagacaagaccatct

SEQ ID NO: 92 - RNA, 21 nt, synthetic construct
  source 1..21: mol_type = other RNA
agatggtcttgtctgtctgga

SEQ ID NO: 93 - RNA, 19 nt, synthetic construct
  source 1..19: mol_type = other RNA
cagacagacaagaccatct

SEQ ID NO: 94 - RNA, 21 nt, synthetic construct
  source 1..21: mol_type = other RNA
agatggtcttgtctgtctgga

SEQ ID NO: 95 - RNA, 19 nt, synthetic construct
  source 1..19: mol_type = other RNA
cagacagacaagaccatct

SEQ ID NO: 96 - RNA, 21 nt, synthetic construct
  source 1..21: mol_type = other RNA
agatggtcttgtctgtctgga

SEQ ID NO: 97 - RNA, 19 nt, synthetic construct
  source 1..19: mol_type = other RNA
cagacagacaagaccatct

SEQ ID NO: 98 - RNA, 21 nt, synthetic construct
  source 1..21: mol_type = other RNA
agatggtcttgtctgtctgga

SEQ ID NO: 99 - RNA, 19 nt, synthetic construct
  source 1..19: mol_type = other RNA
cagacagacaagaccatct

SEQ ID NO: 100 - RNA, 21 nt, synthetic construct
  source 1..21: mol_type = other RNA
agatggtcttgtctgtctgga

SEQ ID NO: 101 - RNA, 19 nt, synthetic construct
  source 1..19: mol_type = other RNA
cagacagacaagaccatct

SEQ ID NO: 102 - RNA, 21 nt, synthetic construct
  source 1..21: mol_type = other RNA
agatggtcttgtctgtctgga

SEQ ID NO: 103 - RNA, 19 nt, synthetic construct
  source 1..19: mol_type = other RNA
cagacagacaagaccatct

SEQ ID NO: 104 - RNA, 21 nt, synthetic construct
  source 1..21: mol_type = other RNA
agatggtcttgtctgtctgga

SEQ ID NO: 105 - RNA, 19 nt, synthetic construct
  source 1..19: mol_type = other RNA
cagacagacaagaccatct

SEQ ID NO: 106 - RNA, 21 nt, synthetic construct
  source 1..21: mol_type = other RNA
agatggtcttgtctgtctgga

SEQ ID NO: 107 - RNA, 19 nt, synthetic construct
  source 1..19: mol_type = other RNA
cagacagacaagaccatct

SEQ ID NO: 108 - RNA, 21 nt, synthetic construct
  source 1..21: mol_type = other RNA
agatggtcttgtctgtctgga

SEQ ID NO: 109 - RNA, 19 nt, synthetic construct
  source 1..19: mol_type = other RNA
cagacagacaagaccatct

SEQ ID NO: 110 - RNA, 21 nt, synthetic construct
  source 1..21: mol_type = other RNA
agatggtcttgtctgtctgga

SEQ ID NO: 111 - RNA, 19 nt, synthetic construct
  source 1..19: mol_type = other RNA
cagacagacaagaccatct

SEQ ID NO: 112 - RNA, 21 nt, synthetic construct
  source 1..21: mol_type = other RNA
agatggtcttgtctgtctgga

SEQ ID NO: 113 - RNA, 19 nt, synthetic construct
  source 1..19: mol_type = other RNA
cagacagacaagaccatct

SEQ ID NO: 114 - RNA, 21 nt, synthetic construct
  source 1..21: mol_type = other RNA
agatggtcttgtctgtctgga

SEQ ID NO: 115 - RNA, 19 nt, synthetic construct
  source 1..19: mol_type = other RNA
cagacagacaagaccatct

SEQ ID NO: 116 - RNA, 21 nt, synthetic construct
  source 1..21: mol_type = other RNA
agatggtcttgtctgtctgga

SEQ ID NO: 117 - RNA, 19 nt, synthetic construct
  source 1..19: mol_type = other RNA
cagacagacaagaccatct

SEQ ID NO: 118 - RNA, 21 nt, synthetic construct
  source 1..21: mol_type = other RNA
agatggtcttgtctgtctgga

SEQ ID NO: 119 - RNA, 19 nt, synthetic construct
  source 1..19: mol_type = other RNA
cagacagacaagaccatct

SEQ ID NO: 120 - RNA, 21 nt, synthetic construct
  source 1..21: mol_type = other RNA
agatggtcttgtctgtctgga

SEQ ID NO: 121 - RNA, 19 nt, synthetic construct
  source 1..19: mol_type = other RNA
cagacagacaagaccatct

SEQ ID NO: 122 - RNA, 21 nt, synthetic construct
  source 1..21: mol_type = other RNA
agatggtcttgtctgtctgga

SEQ ID NO: 123 - RNA, 19 nt, synthetic construct
  source 1..19: mol_type = other RNA
cagacagacaagaccatct

SEQ ID NO: 124 - RNA, 21 nt, synthetic construct
  source 1..21: mol_type = other RNA
agatggtcttgtctgtctgga

SEQ ID NO: 125 - RNA, 19 nt, synthetic construct
  source 1..19: mol_type = other RNA
cagacagacaagaccatct

SEQ ID NO: 126 - RNA, 21 nt, synthetic construct
  source 1..21: mol_type = other RNA
agatggtcttgtctgtctgga

SEQ ID NO: 127 - RNA, 19 nt, synthetic construct
  source 1..19: mol_type = other RNA
cagacagacaagaccatct

SEQ ID NO: 128 - RNA, 21 nt, synthetic construct
  source 1..21: mol_type = other RNA
agatggtcttgtctgtctgga

SEQ ID NO: 129 - RNA, 19 nt, synthetic construct
  source 1..19: mol_type = other RNA
cagacagacaagaccatct

SEQ ID NO: 130 - RNA, 21 nt, synthetic construct
  source 1..21: mol_type = other RNA
agatggtcttgtctgtctgga

SEQ ID NO: 131 - RNA, 19 nt, synthetic construct
  source 1..19: mol_type = other RNA
cagacagacaagaccatct

SEQ ID NO: 132 - RNA, 21 nt, synthetic construct
  source 1..21: mol_type = other RNA
agatggtcttgtctgtctgga

SEQ ID NO: 133 - RNA, 19 nt, synthetic construct
  source 1..19: mol_type = other RNA
cagacagacaagaccatct

SEQ ID NO: 134 - RNA, 21 nt, synthetic construct
  source 1..21: mol_type = other RNA
agatggtcttgtctgtctgga

SEQ ID NO: 135 - RNA, 19 nt, synthetic construct
  source 1..19: mol_type = other RNA
cagacagacaagaccatct

SEQ ID NO: 136 - RNA, 21 nt, synthetic construct
  source 1..21: mol_type = other RNA
agatggtcttgtctgtctgga

SEQ ID NO: 137 - RNA, 19 nt, synthetic construct
  source 1..19: mol_type = other RNA
cagacagacaagaccatct

SEQ ID NO: 138 - RNA, 21 nt, synthetic construct
  source 1..21: mol_type = other RNA
agatggtcttgtctgtctgga

SEQ ID NO: 139 - RNA, 19 nt, synthetic construct
  source 1..19: mol_type = other RNA
cagacagacaagaccatct

SEQ ID NO: 140 - RNA, 21 nt, synthetic construct
  source 1..21: mol_type = other RNA
agatggtcttgtctgtctgga

SEQ ID NO: 141 - RNA, 19 nt, synthetic construct
  source 1..19: mol_type = other RNA
cagacagacaagaccatct

SEQ ID NO: 142 - RNA, 21 nt, synthetic construct
  source 1..21: mol_type = other RNA
agatggtcttgtctgtctgga

SEQ ID NO: 143 - RNA, 19 nt, synthetic construct
  source 1..19: mol_type = other RNA
cagacagacaagaccatct

SEQ ID NO: 144 - RNA, 21 nt, synthetic construct
  source 1..21: mol_type = other RNA
agatggtcttgtctgtctgga

SEQ ID NO: 145 - RNA, 19 nt, synthetic construct
  source 1..19: mol_type = other RNA
cagacagacaagaccatct

SEQ ID NO: 146 - RNA, 21 nt, synthetic construct
  source 1..21: mol_type = other RNA
agatggtcttgtctgtctgga

SEQ ID NO: 147 - RNA, 19 nt, synthetic construct
  source 1..19: mol_type = other RNA
cagacagacaagaccatct

SEQ ID NO: 148 - RNA, 21 nt, synthetic construct
  source 1..21: mol_type = other RNA
agatggtcttgtctgtctgga

SEQ ID NO: 149 - RNA, 19 nt, synthetic construct
  source 1..19: mol_type = other RNA
cagacagacaagaccatct

SEQ ID NO: 150 - RNA, 21 nt, synthetic construct
  source 1..21: mol_type = other RNA
agatggtcttgtctgtctgga

SEQ ID NO: 151 - RNA, 19 nt, synthetic construct
  source 1..19: mol_type = other RNA
cagacagacaagaccatct

SEQ ID NO: 152 - RNA, 21 nt, synthetic construct
  source 1..21: mol_type = other RNA
agatggtcttgtctgtctgga

SEQ ID NO: 153 - RNA, 19 nt, synthetic construct
  source 1..19: mol_type = other RNA
cagacagacaagaccatct

SEQ ID NO: 154 - RNA, 21 nt, synthetic construct
  source 1..21: mol_type = other RNA
agatggtcttgtctgtctgga

SEQ ID NO: 155 - RNA, 19 nt, synthetic construct
  source 1..19: mol_type = other RNA
cagacagacaagaccatct

SEQ ID NO: 156 - RNA, 21 nt, synthetic construct
  source 1..21: mol_type = other RNA
agatggtcttgtctgtctgga

SEQ ID NO: 157 - RNA, 19 nt, synthetic construct
  source 1..19: mol_type = other RNA
cagacagacaagaccatct

SEQ ID NO: 158 - RNA, 21 nt, synthetic construct
  source 1..21: mol_type = other RNA
agatggtcttgtctgtctgga

SEQ ID NO: 159 - RNA, 19 nt, synthetic construct
  source 1..19: mol_type = other RNA
cagacagacaagaccatct

SEQ ID NO: 160 - RNA, 21 nt, synthetic construct
  source 1..21: mol_type = other RNA
agatggtcttgtctgtctgga

SEQ ID NO: 161 - RNA, 19 nt, synthetic construct
  source 1..19: mol_type = other RNA
cagacagacaagaccatct

SEQ ID NO: 162 - RNA, 21 nt, synthetic construct
  source 1..21: mol_type = other RNA
agatggtcttgtctgtctgga

SEQ ID NO: 163 - RNA, 19 nt, synthetic construct
  source 1..19: mol_type = other RNA
cagacagacaagaccatct

SEQ ID NO: 164 - RNA, 21 nt, synthetic construct
  source 1..21: mol_type = other RNA
agatggtcttgtctgtctgga

SEQ ID NO: 165 - RNA, 19 nt, synthetic construct
  source 1..19: mol_type = other RNA
cagacagacaagaccatct

SEQ ID NO: 166 - RNA, 21 nt, synthetic construct
  source 1..21: mol_type = other RNA
agatggtcttgtctgtctgga

SEQ ID NO: 167 - RNA, 19 nt, synthetic construct
  source 1..19: mol_type = other RNA
cagacagacaagaccatct

SEQ ID NO: 168 - RNA, 21 nt, synthetic construct
  source 1..21: mol_type = other RNA
agatggtcttgtctgtctgga

SEQ ID NO: 169 - RNA, 19 nt, synthetic construct
  source 1..19: mol_type = other RNA
cagacagacaagaccatct

SEQ ID NO: 170 - RNA, 21 nt, synthetic construct
  source 1..21: mol_type = other RNA
agatggtcttgtctgtctgga

SEQ ID NO: 171 - RNA, 19 nt, synthetic construct
  source 1..19: mol_type = other RNA
cagacagacaagaccatct

SEQ ID NO: 172 - RNA, 21 nt, synthetic construct
  source 1..21: mol_type = other RNA
agatggtcttgtctgtctgga

SEQ ID NO: 173 - RNA, 19 nt, synthetic construct
  source 1..19: mol_type = other RNA
cagacagacaagaccatct

SEQ ID NO: 174 - RNA, 21 nt, synthetic construct
  source 1..21: mol_type = other RNA
agatggtcttgtctgtctgga

SEQ ID NO: 175 - RNA, 19 nt, synthetic construct
  source 1..19: mol_type = other RNA
ttctccgaacgtgtcacgt

SEQ ID NO: 176 - RNA, 21 nt, synthetic construct
  source 1..21: mol_type = other RNA
acgtgacacgttcggagaact

SEQ ID NO: 177 - RNA, 19 nt, synthetic construct
  source 1..19: mol_type = other RNA
agaagaagatattatctct

SEQ ID NO: 178 - RNA, 21 nt, synthetic construct
  source 1..21: mol_type = other RNA
agagataatatcttcttctgg

SEQ ID NO: 179 - RNA, 19 nt, synthetic construct
  source 1..19: mol_type = other RNA
agaagaagatattatctct

SEQ ID NO: 180 - RNA, 21 nt, synthetic construct
  source 1..21: mol_type = other RNA
agagataatatcttcttctgg

SEQ ID NO: 181 - RNA, 19 nt, synthetic construct
  source 1..19: mol_type = other RNA
agaagaagatattatctct

SEQ ID NO: 182 - RNA, 21 nt, synthetic construct
  source 1..21: mol_type = other RNA
agagataatatcttcttctgg

SEQ ID NO: 183 - RNA, 19 nt, synthetic construct
  source 1..19: mol_type = other RNA
agaagaagatattatctct

SEQ ID NO: 184 - RNA, 21 nt, synthetic construct
  source 1..21: mol_type = other RNA
agagataatatcttcttctgg

SEQ ID NO: 185 - RNA, 19 nt, synthetic construct
  source 1..19: mol_type = other RNA
cagacagacaagaccatct

SEQ ID NO: 186 - RNA, 21 nt, synthetic construct
  source 1..21: mol_type = other RNA
agatggtcttgtctgtctgga

SEQ ID NO: 187 - RNA, 19 nt, synthetic construct
  source 1..19: mol_type = other RNA
cagacagacaagaccatct

SEQ ID NO: 188 - RNA, 21 nt, synthetic construct
  source 1..21: mol_type = other RNA
agatggtcttgtctgtctgga

SEQ ID NO: 189 - RNA, 19 nt, synthetic construct
  source 1..19: mol_type = other RNA
cagacagacaagaccatct

SEQ ID NO: 190 - RNA, 21 nt, synthetic construct
  source 1..21: mol_type = other RNA
agatggtcttgtctgtctgga

SEQ ID NO: 191 - RNA, 19 nt, synthetic construct
  source 1..19: mol_type = other RNA
cagacagacaagaccatct

SEQ ID NO: 192 - RNA, 21 nt, synthetic construct
  source 1..21: mol_type = other RNA
agatggtcttgtctgtctgga

SEQ ID NO: 193 - RNA, 19 nt, synthetic construct
  source 1..19: mol_type = other RNA
cagacagacaagaccatct

SEQ ID NO: 194 - RNA, 21 nt, synthetic construct
  source 1..21: mol_type = other RNA
agatggtcttgtctgtctgga

SEQ ID NO: 195 - RNA, 19 nt, synthetic construct
  source 1..19: mol_type = other RNA
cagacagacaagaccatct

SEQ ID NO: 196 - RNA, 21 nt, synthetic construct
  source 1..21: mol_type = other RNA
agatggtcttgtctgtctgga

SEQ ID NO: 197 - RNA, 19 nt, synthetic construct
  source 1..19: mol_type = other RNA
cagacagacaagaccatct

SEQ ID NO: 198 - RNA, 21 nt, synthetic construct
  source 1..21: mol_type = other RNA
agatggtcttgtctgtctgga

SEQ ID NO: 199 - RNA, 19 nt, synthetic construct
  source 1..19: mol_type = other RNA
cagacagacaagaccatct

SEQ ID NO: 200 - RNA, 21 nt, synthetic construct
  source 1..21: mol_type = other RNA
agatggtcttgtctgtctgga

SEQ ID NO: 201 - RNA, 19 nt, synthetic construct
  source 1..19: mol_type = other RNA
cagacagacaagaccatct

SEQ ID NO: 202 - RNA, 21 nt, synthetic construct
  source 1..21: mol_type = other RNA
agatggtcttgtctgtctgga

SEQ ID NO: 203 - RNA, 19 nt, synthetic construct
  source 1..19: mol_type = other RNA
cagacagacaagaccatct

SEQ ID NO: 204 - RNA, 21 nt, synthetic construct
  source 1..21: mol_type = other RNA
agatggtcttgtctgtctgga

SEQ ID NO: 205 - RNA, 19 nt, synthetic construct
  source 1..19: mol_type = other RNA
cagacagacaagaccatct

SEQ ID NO: 206 - RNA, 21 nt, synthetic construct
  source 1..21: mol_type = other RNA
agatggtcttgtctgtctgga

SEQ ID NO: 207 - RNA, 19 nt, synthetic construct
  source 1..19: mol_type = other RNA
ccaagagcaccaagaacta

SEQ ID NO: 208 - RNA, 21 nt, synthetic construct
  source 1..21: mol_type = other RNA
tagttcttggtgctcttggct

SEQ ID NO: 209 - RNA, 19 nt, synthetic construct
  source 1..19: mol_type = other RNA
ccaagagcaccaagaacta

SEQ ID NO: 210 - RNA, 21 nt, synthetic construct
  source 1..21: mol_type = other RNA
tagttcttggtgctcttggct

SEQ ID NO: 211 - RNA, 19 nt, synthetic construct
  source 1..19: mol_type = other RNA
ccaagagcaccaagaacta

SEQ ID NO: 212 - RNA, 21 nt, synthetic construct
  source 1..21: mol_type = other RNA
tagttcttggtgctcttggct

SEQ ID NO: 213 - RNA, 19 nt, synthetic construct
  source 1..19: mol_type = other RNA
ccaagagcaccaagaacta

SEQ ID NO: 214 - RNA, 21 nt, synthetic construct
  source 1..21: mol_type = other RNA
tagttcttggtgctcttggct

SEQ ID NO: 215 - RNA, 19 nt, synthetic construct
  source 1..19: mol_type = other RNA
ccaagagcaccaagaacta

SEQ ID NO: 216 - RNA, 21 nt, synthetic construct
  source 1..21: mol_type = other RNA
tagttcttggtgctcttggct

SEQ ID NO: 217 - RNA, 19 nt, synthetic construct
  source 1..19: mol_type = other RNA
ccaagagcaccaagaacta

SEQ ID NO: 218 - RNA, 21 nt, synthetic construct
  source 1..21: mol_type = other RNA
tagttcttggtgctcttggct

SEQ ID NO: 219 - RNA, 19 nt, synthetic construct
  source 1..19: mol_type = other RNA
ccaagagcaccaagaacta

SEQ ID NO: 220 - RNA, 21 nt, synthetic construct
  source 1..21: mol_type = other RNA
tagttcttggtgctcttggct

SEQ ID NO: 221 - RNA, 19 nt, synthetic construct
  source 1..19: mol_type = other RNA
ccaagagcaccaagaacta

SEQ ID NO: 222 - RNA, 21 nt, synthetic construct
  source 1..21: mol_type = other RNA
tagttcttggtgctcttggct

SEQ ID NO: 223 - RNA, 19 nt, synthetic construct
  source 1..19: mol_type = other RNA
ccaagagcaccaagaacta

SEQ ID NO: 224 - RNA, 21 nt, synthetic construct
  source 1..21: mol_type = other RNA
tagttcttggtgctcttggct

SEQ ID NO: 225 - RNA, 19 nt, synthetic construct
  source 1..19: mol_type = other RNA
ccaagagcaccaagaacta

SEQ ID NO: 226 - RNA, 21 nt, synthetic construct
  source 1..21: mol_type = other RNA
tagttcttggtgctcttggct

SEQ ID NO: 227 - RNA, 19 nt, synthetic construct
  source 1..19: mol_type = other RNA
ccaagagcaccaagaacta

SEQ ID NO: 228 - RNA, 21 nt, synthetic construct
  source 1..21: mol_type = other RNA
tagttcttggtgctcttggct

SEQ ID NO: 229 - RNA, 19 nt, synthetic construct
  source 1..19: mol_type = other RNA
ccaagagcaccaagaacta

SEQ ID NO: 230 - RNA, 21 nt, synthetic construct
  source 1..21: mol_type = other RNA
tagttcttggtgctcttggct

SEQ ID NO: 231 - RNA, 19 nt, synthetic construct
  source 1..19: mol_type = other RNA
ccaagagcaccaagaacta

SEQ ID NO: 232 - RNA, 21 nt, synthetic construct
  source 1..21: mol_type = other RNA
tagttcttggtgctcttggct

SEQ ID NO: 233 - RNA, 19 nt, synthetic construct
  source 1..19: mol_type = other RNA
ccaagagcaccaagaacta

SEQ ID NO: 234 - RNA, 21 nt, synthetic construct
  source 1..21: mol_type = other RNA
tagttcttggtgctcttggct

SEQ ID NO: 235 - RNA, 19 nt, synthetic construct
  source 1..19: mol_type = other RNA
ccaagagcaccaagaacta

SEQ ID NO: 236 - RNA, 21 nt, synthetic construct
  source 1..21: mol_type = other RNA
tagttcttggtgctcttggct

SEQ ID NO: 237 - RNA, 19 nt, synthetic construct
  source 1..19: mol_type = other RNA
ccaagagcaccaagaacta

SEQ ID NO: 238 - RNA, 21 nt, synthetic construct
  source 1..21: mol_type = other RNA
tagttcttggtgctcttggct

SEQ ID NO: 239 - RNA, 19 nt, synthetic construct
  source 1..19: mol_type = other RNA
ccaagagcaccaagaacta

SEQ ID NO: 240 - RNA, 21 nt, synthetic construct
  source 1..21: mol_type = other RNA
tagttcttggtgctcttggct

SEQ ID NO: 241 - RNA, 19 nt, synthetic construct
  source 1..19: mol_type = other RNA
ccaagagcaccaagaacta

SEQ ID NO: 242 - RNA, 21 nt, synthetic construct
  source 1..21: mol_type = other RNA
tagttcttggtgctcttggct

SEQ ID NO: 243 - RNA, 19 nt, synthetic construct
  source 1..19: mol_type = other RNA
ccaagagcaccaagaacta

SEQ ID NO: 244 - RNA, 21 nt, synthetic construct
  source 1..21: mol_type = other RNA
tagttcttggtgctcttggct

SEQ ID NO: 245 - RNA, 19 nt, synthetic construct
  source 1..19: mol_type = other RNA
ccaagagcaccaagaacta

SEQ ID NO: 246 - RNA, 21 nt, synthetic construct
  source 1..21: mol_type = other RNA
tagttcttggtgctcttggct

SEQ ID NO: 247 - RNA, 19 nt, synthetic construct
  source 1..19: mol_type = other RNA
ccaagagcaccaagaacta

SEQ ID NO: 248 - RNA, 21 nt, synthetic construct
  source 1..21: mol_type = other RNA
tagttcttggtgctcttggct

SEQ ID NO: 249 - RNA, 19 nt, synthetic construct
  source 1..19: mol_type = other RNA
ccaagagcaccaagaacta

SEQ ID NO: 250 - RNA, 21 nt, synthetic construct
  source 1..21: mol_type = other RNA
tagttcttggtgctcttggct

SEQ ID NO: 251 - RNA, 19 nt, synthetic construct
  source 1..19: mol_type = other RNA
ccaagagcaccaagaacta

SEQ ID NO: 252 - RNA, 21 nt, synthetic construct
  source 1..21: mol_type = other RNA
tagttcttggtgctcttggct

SEQ ID NO: 253 - RNA, 19 nt, synthetic construct
  source 1..19: mol_type = other RNA
ccaagagcaccaagaacta

SEQ ID NO: 254 - RNA, 21 nt, synthetic construct
  source 1..21: mol_type = other RNA
tagttcttggtgctcttggtt

SEQ ID NO: 255 - RNA, 19 nt, synthetic construct
  source 1..19: mol_type = other RNA
ccaagagcaccaagaacta

SEQ ID NO: 256 - RNA, 21 nt, synthetic construct
  source 1..21: mol_type = other RNA
tagttcttggtgctcttggct

SEQ ID NO: 257 - RNA, 19 nt, synthetic construct
  source 1..19: mol_type = other RNA
ccaagagcaccaagaacta

SEQ ID NO: 258 - RNA, 21 nt, synthetic construct
  source 1..21: mol_type = other RNA
tagttcttggtgctcttggct

SEQ ID NO: 259 - RNA, 19 nt, synthetic construct
  source 1..19: mol_type = other RNA
ccaagagcaccaagaacta

SEQ ID NO: 260 - RNA, 21 nt, synthetic construct
  source 1..21: mol_type = other RNA
tagttcttggtgctcttggtt

SEQ ID NO: 261 - RNA, 19 nt, synthetic construct
  source 1..19: mol_type = other RNA
ccaagagcaccaagaacta

SEQ ID NO: 262 - RNA, 21 nt, synthetic construct
  source 1..21: mol_type = other RNA
tagttcttggtgctcttggtt

SEQ ID NO: 263 - RNA, 19 nt, synthetic construct
  source 1..19: mol_type = other RNA
ccaagagcaccaagaacta

SEQ ID NO: 264 - RNA, 21 nt, synthetic construct
  source 1..21: mol_type = other RNA
tagttcttggtgctcttggct

SEQ ID NO: 265 - RNA, 19 nt, synthetic construct
  source 1..19: mol_type = other RNA
ccaagagcaccaagaacta

SEQ ID NO: 266 - RNA, 21 nt, synthetic construct
  source 1..21: mol_type = other RNA
tagttcttggtgctcttggct

SEQ ID NO: 267 - RNA, 19 nt, synthetic construct
  source 1..19: mol_type = other RNA
ccaagagcaccaagaacta

SEQ ID NO: 268 - RNA, 21 nt, synthetic construct
  source 1..21: mol_type = other RNA
tagttcttggtgctcttggct

SEQ ID NO: 269 - RNA, 19 nt, synthetic construct
  source 1..19: mol_type = other RNA
ccaagagcaccaagaacta

SEQ ID NO: 270 - RNA, 21 nt, synthetic construct
  source 1..21: mol_type = other RNA
tagttcttggtgctcttggct

SEQ ID NO: 271 - RNA, 19 nt, synthetic construct
  source 1..19: mol_type = other RNA
ccaagagcaccaagaacta

SEQ ID NO: 272 - RNA, 21 nt, synthetic construct
  source 1..21: mol_type = other RNA
tagttcttggtgctcttggct

SEQ ID NO: 273 - RNA, 19 nt, synthetic construct
  source 1..19: mol_type = other RNA
ccaagagcaccaagaacta

SEQ ID NO: 274 - RNA, 21 nt, synthetic construct
  source 1..21: mol_type = other RNA
tagttcttggtgctcttggct

SEQ ID NO: 275 - RNA, 19 nt, synthetic construct
  source 1..19: mol_type = other RNA
ccaagagcaccaagaacta

SEQ ID NO: 276 - RNA, 21 nt, synthetic construct
  source 1..21: mol_type = other RNA
tagttcttggtgctcttggct

SEQ ID NO: 277 - RNA, 21 nt, synthetic construct
  source 1..21: mol_type = other RNA
tagttcttggtgctcttggct

SEQ ID NO: 278 - RNA, 21 nt, synthetic construct
  source 1..21: mol_type = other RNA
tagttcttggtgctcttggct

SEQ ID NO: 279 - RNA, 19 nt, synthetic construct
  source 1..19: mol_type = other RNA
ccaagagcaccaagaacta

SEQ ID NO: 280 - RNA, 21 nt, synthetic construct
  source 1..21: mol_type = other RNA
tagttcttggtgctcttggct

SEQ ID NO: 281 - RNA, 19 nt, synthetic construct
  source 1..19: mol_type = other RNA
ccaagagcaccaagaacta

SEQ ID NO: 282 - RNA, 21 nt, synthetic construct
  source 1..21: mol_type = other RNA
tagttcttggtgctcttggct

SEQ ID NO: 283 - RNA, 19 nt, synthetic construct
  source 1..19: mol_type = other RNA
ccaagagcaccaagaacta

SEQ ID NO: 284 - RNA, 21 nt, synthetic construct
  source 1..21: mol_type = other RNA
tagttcttggtgctcttggct

SEQ ID NO: 285 - RNA, 19 nt, synthetic construct
  source 1..19: mol_type = other RNA
ccaagagcaccaagaacta

SEQ ID NO: 286 - RNA, 21 nt, synthetic construct
  source 1..21: mol_type = other RNA
tagttcttggtgctcttggct

SEQ ID NO: 287 - RNA, 19 nt, synthetic construct
  source 1..19: mol_type = other RNA
ccaagagcaccaagaacta

SEQ ID NO: 288 - RNA, 21 nt, synthetic construct
  source 1..21: mol_type = other RNA
tagttcttggtgctcttggct

SEQ ID NO: 289 - RNA, 19 nt, synthetic construct
  source 1..19: mol_type = other RNA
gtacgtggactggattctg

SEQ ID NO: 290 - RNA, 21 nt, synthetic construct
  source 1..21: mol_type = other RNA
cagaatccagtccacgtactt

SEQ ID NO: 291 - RNA, 19 nt, synthetic construct
  source 1..19: mol_type = other RNA
gtacgtggactggattctg

SEQ ID NO: 292 - RNA, 21 nt, synthetic construct
  source 1..21: mol_type = other RNA
cagaatccagtccacgtactt

SEQ ID NO: 293 - RNA, 19 nt, synthetic construct
  source 1..19: mol_type = other RNA
gtacgtggactggattctg

SEQ ID NO: 294 - RNA, 21 nt, synthetic construct
  source 1..21: mol_type = other RNA
cagaatccagtccacgtactt

SEQ ID NO: 295 - RNA, 19 nt, synthetic construct
  source 1..19: mol_type = other RNA
gtacgtggactggattctg

SEQ ID NO: 296 - RNA, 21 nt, synthetic construct
  source 1..21: mol_type = other RNA
cagaatccagtccacgtactt

SEQ ID NO: 297 - RNA, 19 nt, synthetic construct
  source 1..19: mol_type = other RNA
gtacgtggactggattctg

SEQ ID NO: 298 - RNA, 21 nt, synthetic construct
  source 1..21: mol_type = other RNA
cagaatccagtccacgtactt

SEQ ID NO: 299 - RNA, 19 nt, synthetic construct
  source 1..19: mol_type = other RNA
gtacgtggactggattctg

SEQ ID NO: 300 - RNA, 21 nt, synthetic construct
  source 1..21: mol_type = other RNA
cagaatccagtccacgtactt

SEQ ID NO: 301 - RNA, 19 nt, synthetic construct
  source 1..19: mol_type = other RNA
gtacgtggactggattctg

SEQ ID NO: 302 - RNA, 21 nt, synthetic construct
  source 1..21: mol_type = other RNA
cagaatccagtccacgtactt

SEQ ID NO: 303 - RNA, 19 nt, synthetic construct
  source 1..19: mol_type = other RNA
gtacgtggactggattctg

SEQ ID NO: 304 - RNA, 21 nt, synthetic construct
  source 1..21: mol_type = other RNA
cagaatccagtccacgtactt

SEQ ID NO: 305 - RNA, 19 nt, synthetic construct
  source 1..19: mol_type = other RNA
gtacgtggactggattctg

SEQ ID NO: 306 - RNA, 21 nt, synthetic construct
  source 1..21: mol_type = other RNA
cagaatccagtccacgtactt

SEQ ID NO: 307 - RNA, 19 nt, synthetic construct
  source 1..19: mol_type = other RNA
gtacgtggactggattctg

SEQ ID NO: 308 - RNA, 21 nt, synthetic construct
  source 1..21: mol_type = other RNA
cagaatccagtccacgtactt

SEQ ID NO: 309 - RNA, 19 nt, synthetic construct
  source 1..19: mol_type = other RNA
gtacgtggactggattctg

SEQ ID NO: 310 - RNA, 21 nt, synthetic construct
  source 1..21: mol_type = other RNA
cagaatccagtccacgtactt

SEQ ID NO: 311 - RNA, 19 nt, synthetic construct
  source 1..19: mol_type = other RNA
gtacgtggactggattctg

SEQ ID NO: 312 - RNA, 21 nt, synthetic construct
  source 1..21: mol_type = other RNA
cagaatccagtccacgtactt

SEQ ID NO: 313 - RNA, 19 nt, synthetic construct
  source 1..19: mol_type = other RNA
gtacgtggactggattctg

SEQ ID NO: 314 - RNA, 21 nt, synthetic construct
  source 1..21: mol_type = other RNA
cagaatccagtccacgtactt

SEQ ID NO: 315 - RNA, 19 nt, synthetic construct
  source 1..19: mol_type = other RNA
gtacgtggactggattctg

SEQ ID NO: 316 - RNA, 21 nt, synthetic construct
  source 1..21: mol_type = other RNA
cagaatccagtccacgtactt

SEQ ID NO: 317 - RNA, 19 nt, synthetic construct
  source 1..19: mol_type = other RNA
gtacgtggactggattctg

SEQ ID NO: 318 - RNA, 21 nt, synthetic construct
  source 1..21: mol_type = other RNA
cagaatccagtccacgtactt

SEQ ID NO: 319 - RNA, 19 nt, synthetic construct
  source 1..19: mol_type = other RNA
gtacgtggactggattctg

SEQ ID NO: 320 - RNA, 21 nt, synthetic construct
  source 1..21: mol_type = other RNA
cagaatccagtccacgtactt

SEQ ID NO: 321 - RNA, 19 nt, synthetic construct
  source 1..19: mol_type = other RNA
gtacgtggactggattctg

SEQ ID NO: 322 - RNA, 21 nt, synthetic construct
  source 1..21: mol_type = other RNA
cagaatccagtccacgtactt

SEQ ID NO: 323 - RNA, 19 nt, synthetic construct
  source 1..19: mol_type = other RNA
gtacgtggactggattctg

SEQ ID NO: 324 - RNA, 21 nt, synthetic construct
  source 1..21: mol_type = other RNA
cagaatccagtccacgtactt

SEQ ID NO: 325 - RNA, 19 nt, synthetic construct
  source 1..19: mol_type = other RNA
gtacgtggactggattctg

SEQ ID NO: 326 - RNA, 21 nt, synthetic construct
  source 1..21: mol_type = other RNA
cagaatccagtccacgtactt

SEQ ID NO: 327 - RNA, 19 nt, synthetic construct
  source 1..19: mol_type = other RNA
gtacgtggactggattctg

SEQ ID NO: 328 - RNA, 21 nt, synthetic construct
  source 1..21: mol_type = other RNA
cagaatccagtccacgtactt

SEQ ID NO: 329 - RNA, 19 nt, synthetic construct
  source 1..19: mol_type = other RNA
gtacgtggactggattctg

SEQ ID NO: 330 - RNA, 21 nt, synthetic construct
  source 1..21: mol_type = other RNA
cagaatccagtccacgtactt

SEQ ID NO: 331 - RNA, 19 nt, synthetic construct
  source 1..19: mol_type = other RNA
gtacgtggactggattctg

SEQ ID NO: 332 - RNA, 21 nt, synthetic construct
  source 1..21: mol_type = other RNA
cagaatccagtccacgtactt

SEQ ID NO: 333 - RNA, 19 nt, synthetic construct
  source 1..19: mol_type = other RNA
gtacgtggactggattctg

SEQ ID NO: 334 - RNA, 21 nt, synthetic construct
  source 1..21: mol_type = other RNA
cagaatccagtccacgtactt

SEQ ID NO: 335 - RNA, 19 nt, synthetic construct
  source 1..19: mol_type = other RNA
gtacgtggactggattctg

SEQ ID NO: 336 - RNA, 21 nt, synthetic construct
  source 1..21: mol_type = other RNA
cagaatccagtccacgtactt

SEQ ID NO: 337 - RNA, 19 nt, synthetic construct
  source 1..19: mol_type = other RNA
gtacgtggactggattctg

SEQ ID NO: 338 - RNA, 21 nt, synthetic construct
  source 1..21: mol_type = other RNA
cagaatccagtccacgtactt

SEQ ID NO: 339 - RNA, 19 nt, synthetic construct
  source 1..19: mol_type = other RNA
gtacgtggactggattctg

SEQ ID NO: 340 - RNA, 21 nt, synthetic construct
  source 1..21: mol_type = other RNA
cagaatccagtccacgtactt

SEQ ID NO: 341 - RNA, 19 nt, synthetic construct
  source 1..19: mol_type = other RNA
gtacgtggactggattctg

SEQ ID NO: 342 - RNA, 21 nt, synthetic construct
  source 1..21: mol_type = other RNA
cagaatccagtccacgtactt

SEQ ID NO: 343 - RNA, 19 nt, synthetic construct
  source 1..19: mol_type = other RNA
gtacgtggactggattctg

SEQ ID NO: 344 - RNA, 21 nt, synthetic construct
  source 1..21: mol_type = other RNA
cagaatccagtccacgtactt

SEQ ID NO: 345 - RNA, 19 nt, synthetic construct
  source 1..19: mol_type = other RNA
gtacgtggactggattctg

SEQ ID NO: 346 - RNA, 21 nt, synthetic construct
  source 1..21: mol_type = other RNA
cagaatccagtccacgtactt

SEQ ID NO: 347 - RNA, 19 nt, synthetic construct
  source 1..19: mol_type = other RNA
gtacgtggactggattctg

SEQ ID NO: 348 - RNA, 21 nt, synthetic construct
  source 1..21: mol_type = other RNA
cagaatccagtccacgtactt

SEQ ID NO: 349 - RNA, 19 nt, synthetic construct
  source 1..19: mol_type = other RNA
gtacgtggactggattctg

SEQ ID NO: 350 - RNA, 21 nt, synthetic construct
  source 1..21: mol_type = other RNA
cagaatccagtccacgtactt

SEQ ID NO: 351 - RNA, 19 nt, synthetic construct
  source 1..19: mol_type = other RNA
gtacgtggactggattctg

SEQ ID NO: 352 - RNA, 21 nt, synthetic construct
  source 1..21: mol_type = other RNA
cagaatccagtccacgtactt

SEQ ID NO: 353 - RNA, 19 nt, synthetic construct
  source 1..19: mol_type = other RNA
gtacgtggactggattctg

SEQ ID NO: 354 - RNA, 21 nt, synthetic construct
  source 1..21: mol_type = other RNA
cagaatccagtccacgtactt

SEQ ID NO: 355 - RNA, 19 nt, synthetic construct
  source 1..19: mol_type = other RNA
gtacgtggactggattctg

SEQ ID NO: 356 - RNA, 21 nt, synthetic construct
  source 1..21: mol_type = other RNA
cagaatccagtccacgtactt

SEQ ID NO: 357 - RNA, 19 nt, synthetic construct
  source 1..19: mol_type = other RNA
gtacgtggactggattctg

SEQ ID NO: 358 - RNA, 21 nt, synthetic construct
  source 1..21: mol_type = other RNA
cagaatccagtccacgtactt

SEQ ID NO: 359 - RNA, 19 nt, synthetic construct
  source 1..19: mol_type = other RNA
gtacgtggactggattctg

SEQ ID NO: 360 - RNA, 21 nt, synthetic construct
  source 1..21: mol_type = other RNA
cagaatccagtccacgtactt

SEQ ID NO: 361 - RNA, 19 nt, synthetic construct
  source 1..19: mol_type = other RNA
gtacgtggactggattctg

SEQ ID NO: 362 - RNA, 21 nt, synthetic construct
  source 1..21: mol_type = other RNA
cagaatccagtccacgtactt

SEQ ID NO: 363 - RNA, 19 nt, synthetic construct
  source 1..19: mol_type = other RNA
gtacgtggactggattctg

SEQ ID NO: 364 - RNA, 21 nt, synthetic construct
  source 1..21: mol_type = other RNA
cagaatccagtccacgtactt

SEQ ID NO: 365 - RNA, 19 nt, synthetic construct
  source 1..19: mol_type = other RNA
gtacgtggactggattctg

SEQ ID NO: 366 - RNA, 21 nt, synthetic construct
  source 1..21: mol_type = other RNA
cagaatccagtccacgtactt

SEQ ID NO: 367 - RNA, 19 nt, synthetic construct
  source 1..19: mol_type = other RNA
gtacgtggactggattctg

SEQ ID NO: 368 - RNA, 21 nt, synthetic construct
  source 1..21: mol_type = other RNA
cagaatccagtccacgtactt

SEQ ID NO: 369 - RNA, 19 nt, synthetic construct
  source 1..19: mol_type = other RNA
gtacgtggactggattctg

SEQ ID NO: 370 - RNA, 21 nt, synthetic construct
  source 1..21: mol_type = other RNA
cagaatccagtccacgtactt

SEQ ID NO: 371 - RNA, 19 nt, synthetic construct
  source 1..19: mol_type = other RNA
ttttaatcctcactctaaa

SEQ ID NO: 372 - RNA, 21 nt, synthetic construct
  source 1..21: mol_type = other RNA
tttagagtgaggattaaaatg

SEQ ID NO: 373 - RNA, 19 nt, synthetic construct
  source 1..19: mol_type = other RNA
ttttaatcctcactctaaa

SEQ ID NO: 374 - RNA, 21 nt, synthetic construct
  source 1..21: mol_type = other RNA
tttagagtgaggattaaaatg

SEQ ID NO: 375 - RNA, 19 nt, synthetic construct
  source 1..19: mol_type = other RNA
ttttaatcctcactctaaa

SEQ ID NO: 376 - RNA, 21 nt, synthetic construct
  source 1..21: mol_type = other RNA
tttagagtgaggattaaaatg

SEQ ID NO: 377 - RNA, 19 nt, synthetic construct
  source 1..19: mol_type = other RNA
ttttaatcctcactctaaa

SEQ ID NO: 378 - RNA, 21 nt, synthetic construct
  source 1..21: mol_type = other RNA
tttagagtgaggattaaaatg

SEQ ID NO: 379 - RNA, 19 nt, synthetic construct
  source 1..19: mol_type = other RNA
ttttaatcctcactctaaa

SEQ ID NO: 380 - RNA, 21 nt, synthetic construct
  source 1..21: mol_type = other RNA
tttagagtgaggattaaaatg

SEQ ID NO: 381 - RNA, 19 nt, synthetic construct
  source 1..19: mol_type = other RNA
ttttaatcctcactctaaa

SEQ ID NO: 382 - RNA, 21 nt, synthetic construct
  source 1..21: mol_type = other RNA
tttagagtgaggattaaaatg

SEQ ID NO: 383 - RNA, 19 nt, synthetic construct
  source 1..19: mol_type = other RNA
ttttaatcctcactctaaa

SEQ ID NO: 384 - RNA, 21 nt, synthetic construct
  source 1..21: mol_type = other RNA
tttagagtgaggattaaaatg

SEQ ID NO: 385 - RNA, 19 nt, synthetic construct
  source 1..19: mol_type = other RNA
ttttaatcctcactctaaa

SEQ ID NO: 386 - RNA, 21 nt, synthetic construct
  source 1..21: mol_type = other RNA
tttagagtgaggattaaaatg

SEQ ID NO: 387 - RNA, 19 nt, synthetic construct
  source 1..19: mol_type = other RNA
ttttaatcctcactctaaa

SEQ ID NO: 388 - RNA, 20 nt, synthetic construct
  source 1..20: mol_type = other RNA
tttagaggaggattaaaatg

SEQ ID NO: 389 - RNA, 19 nt, synthetic construct
  source 1..19: mol_type = other RNA
ttttaatcctcactctaaa

SEQ ID NO: 390 - RNA, 20 nt, synthetic construct
  source 1..20: mol_type = other RNA
tttagagtgaggataaaatg

SEQ ID NO: 391 - RNA, 19 nt, synthetic construct
  source 1..19: mol_type = other RNA
ttttaatcctcactctaaa

SEQ ID NO: 392 - RNA, 20 nt, synthetic construct
  source 1..20: mol_type = other RNA
tttagaggaggattaaaatg

SEQ ID NO: 393 - RNA, 19 nt, synthetic construct
  source 1..19: mol_type = other RNA
ttttaatcctcactctaaa

SEQ ID NO: 394 - RNA, 20 nt, synthetic construct
  source 1..20: mol_type = other RNA
tttagagtgaggataaaatg

SEQ ID NO: 395 - DNA, 20 bp, synthetic construct
  source 1..20: mol_type = other DNA
aagcgcattccgattgagga

SEQ ID NO: 396 - DNA, 20 bp, synthetic construct
  source 1..20: mol_type = other DNA
cctgagtgcaagatgacggt

SEQ ID NO: 397 - DNA, 19 bp, synthetic construct
  source 1..19: mol_type = other DNA
ggtcggagtcaacggattt

SEQ ID NO: 398 - DNA, 19 bp, synthetic construct
  source 1..19: mol_type = other DNA
ccagcatcgccccacttga

SEQ ID NO: 399 - DNA, 23 bp, synthetic construct
  source 1..23: mol_type = other DNA
gaggagcagctaaccaacttaat

SEQ ID NO: 400 - DNA, 23 bp, synthetic construct
  source 1..23: mol_type = other DNA
tctgcatgtgctgttgacttaat

SEQ ID NO: 401 - DNA, 19 bp, synthetic construct
  source 1..19: mol_type = other DNA
tgcaccaccaactgcttag

SEQ ID NO: 402 - DNA, 19 bp, synthetic construct
  source 1..19: mol_type = other DNA
ggatgcagggatgatgttc

SEQ ID NO: 403 - DNA, 23 bp, synthetic construct
  source 1..23: mol_type = other DNA
gccctgttaaaactggaatcagc

SEQ ID NO: 404 - DNA, 23 bp, synthetic construct
  source 1..23: mol_type = other DNA
gccctgttaaaactggaatcagc

SEQ ID NO: 405 - DNA, 19 bp, synthetic construct
  source 1..19: mol_type = other DNA
tgcaccaccaactgcttag

SEQ ID NO: 406 - DNA, 19 bp, synthetic construct
  source 1..19: mol_type = other DNA
ggatgcagggatgatgttc

SEQ ID NO: 407 - RNA, 19 nt, synthetic construct
  source 1..19: mol_type = other RNA
cagagaaattctactacat

SEQ ID NO: 408 - RNA, 21 nt, synthetic construct
  source 1..21: mol_type = other RNA
atgtagtagaatttctctgta

SEQ ID NO: 409 - RNA, 19 nt, synthetic construct
  source 1..19: mol_type = other RNA
cagagaaattctactacat

SEQ ID NO: 410 - RNA, 21 nt, synthetic construct
  source 1..21: mol_type = other RNA
atgtagtagaatttctctgta

SEQ ID NO: 411 - RNA, 19 nt, synthetic construct
  source 1..19: mol_type = other RNA
cagagaaattctactacat

SEQ ID NO: 412 - RNA, 21 nt, synthetic construct
  source 1..21: mol_type = other RNA
atgtagtagaatttctctgta

SEQ ID NO: 413 - RNA, 19 nt, synthetic construct
  source 1..19: mol_type = other RNA
cagagaaattctactacat

SEQ ID NO: 414 - RNA, 21 nt, synthetic construct
  source 1..21: mol_type = other RNA
atgtagtagaatttctctgta

SEQ ID NO: 415 - RNA, 19 nt, synthetic construct
  source 1..19: mol_type = other RNA
cagagaaattctactacat

SEQ ID NO: 416 - RNA, 21 nt, synthetic construct
  source 1..21: mol_type = other RNA
atgtagtagaatttctctgta

SEQ ID NO: 417 - RNA, 19 nt, synthetic construct
  source 1..19: mol_type = other RNA
cagagaaattctactacat

SEQ ID NO: 418 - RNA, 21 nt, synthetic construct
  source 1..21: mol_type = other RNA
atgtagtagaatttctctgta

SEQ ID NO: 419 - RNA, 19 nt, synthetic construct
  source 1..19: mol_type = other RNA
cagagaaattctactacat

SEQ ID NO: 420 - RNA, 21 nt, synthetic construct
  source 1..21: mol_type = other RNA
atgtagtagaatttctctgta

SEQ ID NO: 421 - RNA, 19 nt, synthetic construct
  source 1..19: mol_type = other RNA
cagagaaattctactacat

SEQ ID NO: 422 - RNA, 21 nt, synthetic construct
  source 1..21: mol_type = other RNA
atgtagtagaatttctctgta

SEQ ID NO: 423 - RNA, 19 nt, synthetic construct
  source 1..19: mol_type = other RNA
cagagaaattctactacat

SEQ ID NO: 424 - RNA, 21 nt, synthetic construct
  source 1..21: mol_type = other RNA
atgtagtagaatttctctgta

SEQ ID NO: 425 - RNA, 19 nt, synthetic construct
  source 1..19: mol_type = other RNA
cgaagctcatgaatatatt

SEQ ID NO: 426 - RNA, 21 nt, synthetic construct
  source 1..21: mol_type = other RNA
aatatattcatgagcttcgta

SEQ ID NO: 427 - RNA, 19 nt, synthetic construct
  source 1..19: mol_type = other RNA
cgaagctcatgaatatatt

SEQ ID NO: 428 - RNA, 21 nt, synthetic construct
  source 1..21: mol_type = other RNA
aatatattcatgagcttcgta

SEQ ID NO: 429 - RNA, 19 nt, synthetic construct
  source 1..19: mol_type = other RNA
cgaagctcatgaatatatt

SEQ ID NO: 430 - RNA, 21 nt, synthetic construct
  source 1..21: mol_type = other RNA
aatatattcatgagcttcgta

SEQ ID NO: 431 - RNA, 19 nt, synthetic construct
  source 1..19: mol_type = other RNA
cgaagctcatgaatatatt

SEQ ID NO: 432 - RNA, 21 nt, synthetic construct
  source 1..21: mol_type = other RNA
aatatattcatgagcttcgta

SEQ ID NO: 433 - RNA, 19 nt, synthetic construct
  source 1..19: mol_type = other RNA
cgaagctcatgaatatatt

SEQ ID NO: 434 - RNA, 21 nt, synthetic construct
  source 1..21: mol_type = other RNA
aatatattcatgagcttcgta

SEQ ID NO: 435 - RNA, 19 nt, synthetic construct
  source 1..19: mol_type = other RNA
cgaagctcatgaatatatt

SEQ ID NO: 436 - RNA, 21 nt, synthetic construct
  source 1..21: mol_type = other RNA
aatatattcatgagcttcgta

SEQ ID NO: 437 - RNA, 19 nt, synthetic construct
  source 1..19: mol_type = other RNA
cgaagctcatgaatatatt

SEQ ID NO: 438 - RNA, 21 nt, synthetic construct
  source 1..21: mol_type = other RNA
aatatattcatgagcttcgta

SEQ ID NO: 439 - RNA, 19 nt, synthetic construct
  source 1..19: mol_type = other RNA
cgaagctcatgaatatatt

SEQ ID NO: 440 - RNA, 21 nt, synthetic construct
  source 1..21: mol_type = other RNA
aatatattcatgagcttcgta

SEQ ID NO: 441 - RNA, 19 nt, synthetic construct
  source 1..19: mol_type = other RNA
cgaagctcatgaatatatt

SEQ ID NO: 442 - RNA, 21 nt, synthetic construct
  source 1..21: mol_type = other RNA
aatatattcatgagcttcgta

SEQ ID NO: 443 - RNA, 19 nt, synthetic construct
  source 1..19: mol_type = other RNA
cgaagctcatgaatatatt

SEQ ID NO: 444 - RNA, 21 nt, synthetic construct
  source 1..21: mol_type = other RNA
aatatattcatgagcttcgta

SEQ ID NO: 445 - RNA, 19 nt, synthetic construct
  source 1..19: mol_type = other RNA
gagaattgcttcatacaaa

SEQ ID NO: 446 - RNA, 21 nt, synthetic construct
  source 1..21: mol_type = other RNA
tttgtatgaagcaattctcct

SEQ ID NO: 447 - RNA, 19 nt, synthetic construct
  source 1..19: mol_type = other RNA
gagaattgcttcatacaaa

SEQ ID NO: 448 - RNA, 21 nt, synthetic construct
  source 1..21: mol_type = other RNA
tttgtatgaagcaattctcct

SEQ ID NO: 449 - RNA, 19 nt, synthetic construct
  source 1..19: mol_type = other RNA
gagaattgcttcatacaaa

SEQ ID NO: 450 - RNA, 21 nt, synthetic construct
  source 1..21: mol_type = other RNA
tttgtatgaagcaattctcct

SEQ ID NO: 451 - RNA, 19 nt, synthetic construct
  source 1..19: mol_type = other RNA
gagaattgcttcatacaaa

SEQ ID NO: 452 - RNA, 21 nt, synthetic construct
  source 1..21: mol_type = other RNA
tttgtatgaagcaattctcct

SEQ ID NO: 453 - RNA, 19 nt, synthetic construct
  source 1..19: mol_type = other RNA
gagaattgcttcatacaaa

SEQ ID NO: 454 - RNA, 21 nt, synthetic construct
  source 1..21: mol_type = other RNA
tttgtatgaagcaattctcct

SEQ ID NO: 455 - RNA, 19 nt, synthetic construct
  source 1..19: mol_type = other RNA
gagaattgcttcatacaaa

SEQ ID NO: 456 - RNA, 21 nt, synthetic construct
  source 1..21: mol_type = other RNA
tttgtatgaagcaattctcct

SEQ ID NO: 457 - RNA, 19 nt, synthetic construct
  source 1..19: mol_type = other RNA
caactcacctgtaataaat

SEQ ID NO: 458 - RNA, 21 nt, synthetic construct
  source 1..21: mol_type = other RNA
atttattacaggtgagttgat

SEQ ID NO: 459 - RNA, 19 nt, synthetic construct
  source 1..19: mol_type = other RNA
caactcacctgtaataaat

SEQ ID NO: 460 - RNA, 21 nt, synthetic construct
  source 1..21: mol_type = other RNA
atttattacaggtgagttgat

SEQ ID NO: 461 - RNA, 19 nt, synthetic construct
  source 1..19: mol_type = other RNA
caactcacctgtaataaat

SEQ ID NO: 462 - RNA, 21 nt, synthetic construct
  source 1..21: mol_type = other RNA
atttattacaggtgagttgat

SEQ ID NO: 463 - RNA, 19 nt, synthetic construct
  source 1..19: mol_type = other RNA
caactcacctgtaataaat

SEQ ID NO: 464 - RNA, 21 nt, synthetic construct
  source 1..21: mol_type = other RNA
atttattacaggtgagttgat

SEQ ID NO: 465 - RNA, 19 nt, synthetic construct
  source 1..19: mol_type = other RNA
caactcacctgtaataaat

SEQ ID NO: 466 - RNA, 21 nt, synthetic construct
  source 1..21: mol_type = other RNA
atttattacaggtgagttgat

SEQ ID NO: 467 - RNA, 19 nt, synthetic construct
  source 1..19: mol_type = other RNA
caactcacctgtaataaat

SEQ ID NO: 468 - RNA, 21 nt, synthetic construct
  source 1..21: mol_type = other RNA
atttattacaggtgagttgat

SEQ ID NO: 469 - RNA, 19 nt, synthetic construct
  source 1..19: mol_type = other RNA
caactcacctgtaataaat

SEQ ID NO: 470 - RNA, 21 nt, synthetic construct
  source 1..21: mol_type = other RNA
atttattacaggtgagttgat

SEQ ID NO: 471 - RNA, 19 nt, synthetic construct
  source 1..19: mol_type = other RNA
caactcacctgtaataaat

SEQ ID NO: 472 - RNA, 21 nt, synthetic construct
  source 1..21: mol_type = other RNA
atttattacaggtgagttgat

SEQ ID NO: 473 - RNA, 19 nt, synthetic construct
  source 1..19: mol_type = other RNA
caactcacctgtaataaat

SEQ ID NO: 474 - RNA, 21 nt, synthetic construct
  source 1..21: mol_type = other RNA
atttattacaggtgagttgat

SEQ ID NO: 475 - RNA, 19 nt, synthetic construct
  source 1..19: mol_type = other RNA
cgaagctcatgaatatatt

SEQ ID NO: 476 - RNA, 21 nt, synthetic construct
  source 1..21: mol_type = other RNA
aatatattcatgagcttcgta

SEQ ID NO: 477 - RNA, 19 nt, synthetic construct
  source 1..19: mol_type = other RNA
cgaagctcatgaatatatt

SEQ ID NO: 478 - RNA, 21 nt, synthetic construct
  source 1..21: mol_type = other RNA
aatatattcatgagcttcgta

SEQ ID NO: 479 - RNA, 19 nt, synthetic construct
  source 1..19: mol_type = other RNA
cagagaaattctactacat

SEQ ID NO: 480 - RNA, 21 nt, synthetic construct
  source 1..21: mol_type = other RNA
atgtagtagaatttctctgta

SEQ ID NO: 481 - RNA, 19 nt, synthetic construct
  source 1..19: mol_type = other RNA
caactcacctgtaataaat

SEQ ID NO: 482 - RNA, 21 nt, synthetic construct
  source 1..21: mol_type = other RNA
atttattacaggtgagttgat

SEQ ID NO: 483 - RNA, 19 nt, synthetic construct
  source 1..19: mol_type = other RNA
caagttgagaacaaaaatt

SEQ ID NO: 484 - RNA, 21 nt, synthetic construct
  source 1..21: mol_type = other RNA
aatttttgttctcaacttgaa

SEQ ID NO: 485 - RNA, 19 nt, synthetic construct
  source 1..19: mol_type = other RNA
caagttgagaacaaaaatt

SEQ ID NO: 486 - RNA, 21 nt, synthetic construct
  source 1..21: mol_type = other RNA
aatttttgttctcaacttgaa

SEQ ID NO: 487 - RNA, 19 nt, synthetic construct
  source 1..19: mol_type = other RNA
caagttgagaacaaaaatt

SEQ ID NO: 488 - RNA, 21 nt, synthetic construct
  source 1..21: mol_type = other RNA
aatttttgttctcaacttgaa

SEQ ID NO: 489 - RNA, 19 nt, synthetic construct
  source 1..19: mol_type = other RNA
caagttgagaacaaaaatt

SEQ ID NO: 490 - RNA, 21 nt, synthetic construct
  source 1..21: mol_type = other RNA
aatttttgttctcaacttgaa

SEQ ID NO: 491 - RNA, 19 nt, synthetic construct
  source 1..19: mol_type = other RNA
caagttgagaacaaaaatt

SEQ ID NO: 492 - RNA, 21 nt, synthetic construct
  source 1..21: mol_type = other RNA
aatttttgttctcaacttgaa

SEQ ID NO: 493 - RNA, 19 nt, synthetic construct
  source 1..19: mol_type = other RNA
gttttaaaattaaagtata

SEQ ID NO: 494 - RNA, 21 nt, synthetic construct
  source 1..21: mol_type = other RNA
tatactttaattttaaaaccc

SEQ ID NO: 495 - RNA, 19 nt, synthetic construct
  source 1..19: mol_type = other RNA
gttttaaaattaaagtata

SEQ ID NO: 496 - RNA, 21 nt, synthetic construct
  source 1..21: mol_type = other RNA
tatactttaattttaaaaccc

SEQ ID NO: 497 - RNA, 19 nt, synthetic construct
  source 1..19: mol_type = other RNA
gttttaaaattaaagtata

SEQ ID NO: 498 - RNA, 21 nt, synthetic construct
  source 1..21: mol_type = other RNA
tatactttaattttaaaaccc

SEQ ID NO: 499 - RNA, 19 nt, synthetic construct
  source 1..19: mol_type = other RNA
aagtatacatttttgcatt

SEQ ID NO: 500 - RNA, 21 nt, synthetic construct
  source 1..21: mol_type = other RNA
aatgcaaaaatgtatacttta

SEQ ID NO: 501 - RNA, 19 nt, synthetic construct
  source 1..19: mol_type = other RNA
aagtatacatttttgcatt

SEQ ID NO: 502 - RNA, 21 nt, synthetic construct
  source 1..21: mol_type = other RNA
aatgcaaaaatgtatacttta

SEQ ID NO: 503 - RNA, 19 nt, synthetic construct
  source 1..19: mol_type = other RNA
aagtatacatttttgcatt

SEQ ID NO: 504 - RNA, 21 nt, synthetic construct
  source 1..21: mol_type = other RNA
aatgcaaaaatgtatacttta

SEQ ID NO: 505 - RNA, 19 nt, synthetic construct
  source 1..19: mol_type = other RNA
gttttaaaattaaagtata

SEQ ID NO: 506 - RNA, 21 nt, synthetic construct
  source 1..21: mol_type = other RNA
tatactttaattttaaaaccc

SEQ ID NO: 507 - RNA, 19 nt, synthetic construct
  source 1..19: mol_type = other RNA
ggcttgatcatgaactact

SEQ ID NO: 508 - RNA, 21 nt, synthetic construct
  source 1..21: mol_type = other RNA
agtagttcatgatcaagccag

SEQ ID NO: 509 - RNA, 19 nt, synthetic construct
  source 1..19: mol_type = other RNA
gcagctccttattgttata

SEQ ID NO: 510 - RNA, 21 nt, synthetic construct
  source 1..21: mol_type = other RNA
tataacaataaggagctgcca

SEQ ID NO: 511 - RNA, 19 nt, synthetic construct
  source 1..19: mol_type = other RNA
cggtaatggacagagttat

SEQ ID NO: 512 - RNA, 21 nt, synthetic construct
  source 1..21: mol_type = other RNA
ataactctgtccattaccgtg

SEQ ID NO: 513 - RNA, 19 nt, synthetic construct
  source 1..19: mol_type = other RNA
ctggcttgatcaagaacta

SEQ ID NO: 514 - RNA, 21 nt, synthetic construct
  source 1..21: mol_type = other RNA
tagttcttgatcaagccagca

SEQ ID NO: 515 - RNA, 19 nt, synthetic construct
  source 1..19: mol_type = other RNA
ctgacacaatgctcagaaa

SEQ ID NO: 516 - RNA, 21 nt, synthetic construct
  source 1..21: mol_type = other RNA
tttctgagcattgtgtcagat

SEQ ID NO: 517 - RNA, 19 nt, synthetic construct
  source 1..19: mol_type = other RNA
ggcttgatcatgaactact

SEQ ID NO: 518 - RNA, 21 nt, synthetic construct
  source 1..21: mol_type = other RNA
agtagttcatgatcaagccag

SEQ ID NO: 519 - RNA, 19 nt, synthetic construct
  source 1..19: mol_type = other RNA
gcagctccttattgttata

SEQ ID NO: 520 - RNA, 21 nt, synthetic construct
  source 1..21: mol_type = other RNA
tataacaataaggagctgcca

SEQ ID NO: 521 - RNA, 19 nt, synthetic construct
  source 1..19: mol_type = other RNA
cggtaatggacagagttat

SEQ ID NO: 522 - RNA, 21 nt, synthetic construct
  source 1..21: mol_type = other RNA
ataactctgtccattaccgtg

SEQ ID NO: 523 - RNA, 19 nt, synthetic construct
  source 1..19: mol_type = other RNA
ctggcttgatcaagaacta

SEQ ID NO: 524 - RNA, 21 nt, synthetic construct
  source 1..21: mol_type = other RNA
tagttcttgatcaagccagca

SEQ ID NO: 525 - RNA, 19 nt, synthetic construct
  source 1..19: mol_type = other RNA
ctgacacaatgctcagaaa

SEQ ID NO: 526 - RNA, 21 nt, synthetic construct
  source 1..21: mol_type = other RNA
tttctgagcattgtgtcagat

SEQ ID NO: 527 - RNA, 19 nt, synthetic construct
  source 1..19: mol_type = other RNA
ttttaatcctcactctaaa

SEQ ID NO: 528 - RNA, 21 nt, synthetic construct
  source 1..21: mol_type = other RNA
tttagagtgaggattaaaatg

SEQ ID NO: 529 - RNA, 19 nt, synthetic construct
  source 1..19: mol_type = other RNA
ttttaatcctcactctaaa

SEQ ID NO: 530 - RNA, 21 nt, synthetic construct
  source 1..21: mol_type = other RNA
tttagagtgaggattaaaatg

SEQ ID NO: 531 - RNA, 19 nt, synthetic construct
  source 1..19: mol_type = other RNA
ttttaatcctcactctaaa

SEQ ID NO: 532 - RNA, 21 nt, synthetic construct
  source 1..21: mol_type = other RNA
tttagagtgaggattaaaatg

SEQ ID NO: 533 - RNA, 19 nt, synthetic construct
  source 1..19: mol_type = other RNA
ttttaatcctcactctaaa

SEQ ID NO: 534 - RNA, 21 nt, synthetic construct
  source 1..21: mol_type = other RNA
tttagagtgaggattaaaatg

SEQ ID NO: 535 - RNA, 19 nt, synthetic construct
  source 1..19: mol_type = other RNA
ttttaatcctcactctaaa

SEQ ID NO: 536 - RNA, 21 nt, synthetic construct
  source 1..21: mol_type = other RNA
tttagagtgaggattaaaatg

SEQ ID NO: 537 - RNA, 19 nt, synthetic construct
  source 1..19: mol_type = other RNA
ttttaatcctcactctaaa

SEQ ID NO: 538 - RNA, 21 nt, synthetic construct
  source 1..21: mol_type = other RNA
tttagagtgaggattaaaatg

SEQ ID NO: 539 - RNA, 19 nt, synthetic construct
  source 1..19: mol_type = other RNA
ttttaatcctcactctaaa

SEQ ID NO: 540 - RNA, 21 nt, synthetic construct
  source 1..21: mol_type = other RNA
tttagagtgaggattaaaatg

SEQ ID NO: 541 - RNA, 19 nt, synthetic construct
  source 1..19: mol_type = other RNA
ttttaatcctcactctaaa

SEQ ID NO: 542 - RNA, 21 nt, synthetic construct
  source 1..21: mol_type = other RNA
tttagagtgaggattaaaatg

SEQ ID NO: 543 - RNA, 19 nt, synthetic construct
  source 1..19: mol_type = other RNA
ccaagagcaccaagaacta

SEQ ID NO: 544 - RNA, 21 nt, synthetic construct
  source 1..21: mol_type = other RNA
tagttcttggtgctcttggtt

SEQ ID NO: 545 - RNA, 19 nt, synthetic construct
  source 1..19: mol_type = other RNA
ccaagagcaccaagaacta

SEQ ID NO: 546 - RNA, 21 nt, synthetic construct
  source 1..21: mol_type = other RNA
tagttcttggtgctcttggtt

SEQ ID NO: 547 - RNA, 19 nt, synthetic construct
  source 1..19: mol_type = other RNA
ccaagagcaccaagaacta

SEQ ID NO: 548 - RNA, 21 nt, synthetic construct
  source 1..21: mol_type = other RNA
tagttcttggtgctcttggct

SEQ ID NO: 549 - RNA, 19 nt, synthetic construct
  source 1..19: mol_type = other RNA
gctcaaccaaatcagttat

SEQ ID NO: 550 - RNA, 21 nt, synthetic construct
  source 1..21: mol_type = other RNA
ataactgatttggttgagctt

SEQ ID NO: 551 - RNA, 19 nt, synthetic construct
  source 1..19: mol_type = other RNA
gctcaaccaaatcagttat

SEQ ID NO: 552 - RNA, 21 nt, synthetic construct
  source 1..21: mol_type = other RNA
ataactgatttggttgagctt

SEQ ID NO: 553 - RNA, 19 nt, synthetic construct
  source 1..19: mol_type = other RNA
gctcaaccaaatcagttat

SEQ ID NO: 554 - RNA, 21 nt, synthetic construct
  source 1..21: mol_type = other RNA
ataactgatttggttgagctt

SEQ ID NO: 555 - RNA, 20 nt, synthetic construct
  source 1..20: mol_type = other RNA
gctcaacccaaatcagttat

SEQ ID NO: 556 - RNA, 21 nt, synthetic construct
  source 1..21: mol_type = other RNA
ataactgatttggttgagctt

SEQ ID NO: 557 - RNA, 19 nt, synthetic construct
  source 1..19: mol_type = other RNA
ggagggagtagagatcaaa

SEQ ID NO: 558 - RNA, 21 nt, synthetic construct
  source 1..21: mol_type = other RNA
tttgatctctactccctccag

SEQ ID NO: 559 - RNA, 19 nt, synthetic construct
  source 1..19: mol_type = other RNA
ggagggagtagagatcaaa

SEQ ID NO: 560 - RNA, 21 nt, synthetic construct
  source 1..21: mol_type = other RNA
tttgatctctactccctccag

SEQ ID NO: 561 - RNA, 19 nt, synthetic construct
  source 1..19: mol_type = other RNA
ggagggagtagagatcaaa

SEQ ID NO: 562 - RNA, 21 nt, synthetic construct
  source 1..21: mol_type = other RNA
tttgatctctactccctccag

SEQ ID NO: 563 - RNA, 19 nt, synthetic construct
  source 1..19: mol_type = other RNA
ggagggagtagagatcaaa

SEQ ID NO: 564 - RNA, 21 nt, synthetic construct
  source 1..21: mol_type = other RNA
tttgatctctactccctccag

SEQ ID NO: 565 - RNA, 19 nt, synthetic construct
  source 1..19: mol_type = other RNA
ggagggagtagagatcaaa

SEQ ID NO: 566 - RNA, 21 nt, synthetic construct
  source 1..21: mol_type = other RNA
tttgatctctactccctccag

SEQ ID NO: 567 - RNA, 19 nt, synthetic construct
  source 1..19: mol_type = other RNA
caacagtgatgaaatccaa

SEQ ID NO: 568 - RNA, 21 nt, synthetic construct
  source 1..21: mol_type = other RNA
ttggatttcatcactgttgct

SEQ ID NO: 569 - RNA, 19 nt, synthetic construct
  source 1..19: mol_type = other RNA
caacagtgatgaaatccaa

SEQ ID NO: 570 - RNA, 21 nt, synthetic construct
  source 1..21: mol_type = other RNA
ttggatttcatcactgttgct

SEQ ID NO: 571 - RNA, 19 nt, synthetic construct
  source 1..19: mol_type = other RNA
ccaagagcaccaagaacta

SEQ ID NO: 572 - RNA, 21 nt, synthetic construct
  source 1..21: mol_type = other RNA
tagttcttggtgctcttggtt

SEQ ID NO: 573 - RNA, 19 nt, synthetic construct
  source 1..19: mol_type = other RNA
ccaagagcaccaagaacta

SEQ ID NO: 574 - RNA, 21 nt, synthetic construct
  source 1..21: mol_type = other RNA
tagttcttggtgctcttggtt

SEQ ID NO: 575 - RNA, 19 nt, synthetic construct
  source 1..19: mol_type = other RNA
ccaagagcaccaagaacta

SEQ ID NO: 576 - RNA, 21 nt, synthetic construct
  source 1..21: mol_type = other RNA
tagttcttggtgctcttggtt

SEQ ID NO: 577 - RNA, 19 nt, synthetic construct
  source 1..19: mol_type = other RNA
ttttaatcctcactctaaa

SEQ ID NO: 578 - RNA, 21 nt, synthetic construct
  source 1..21: mol_type = other RNA
tttagagtgaggattaaaatg

SEQ ID NO: 579 - RNA, 19 nt, synthetic construct
  source 1..19: mol_type = other RNA
ttttaatcctcactctaaa

SEQ ID NO: 580 - RNA, 21 nt, synthetic construct
  source 1..21: mol_type = other RNA
tttagagtgaggattaaaatt

SEQ ID NO: 581 - DNA, 21 bp, synthetic construct
  source 1..21: mol_type = other DNA
agtctcctgctttagtgatgc

SEQ ID NO: 582 - DNA, 20 bp, synthetic construct
  source 1..20: mol_type = other DNA
gcctttgttctcatctcgct

SEQ ID NO: 583 - DNA, 27 bp, synthetic construct
  source 1..27: mol_type = other DNA
ctgttgacctgctcctcgcaaatatct

SEQ ID NO: 584 - DNA, 19 bp, synthetic construct
  source 1..19: mol_type = other DNA
aagaaggtggtgaagcagg

SEQ ID NO: 585 - DNA, 18 bp, synthetic construct
  source 1..18: mol_type = other DNA
caaagtggtcgttgaggg

SEQ ID NO: 586 - DNA, 18 bp, synthetic construct
  source 1..18: mol_type = other DNA
caacagcgacacccactc

SEQ ID NO: 587 - DNA, 19 bp, synthetic construct
  source 1..19: mol_type = other DNA
gtatgtacacccggtcacc

SEQ ID NO: 588 - DNA, 21 bp, synthetic construct
  source 1..21: mol_type = other DNA
gttgttctgggtactacagca

SEQ ID NO: 589 - DNA, 21 bp, synthetic construct
  source 1..21: mol_type = other DNA
catcctctgcctcctggcctg

SEQ ID NO: 590 - DNA, 19 bp, synthetic construct
  source 1..19: mol_type = other DNA
aagaaggtggtgaagcagg

SEQ ID NO: 591 - DNA, 18 bp, synthetic construct
  source 1..18: mol_type = other DNA
caaagtggtcgttgaggg

SEQ ID NO: 592 - DNA, 18 bp, synthetic construct
  source 1..18: mol_type = other DNA
caacagcgacacccactc

SEQ ID NO: 593 - DNA, 18 bp, synthetic construct
  source 1..18: mol_type = other DNA
gacacgatgctcagatgc

SEQ ID NO: 594 - DNA, 18 bp, synthetic construct
  source 1..18: mol_type = other DNA
ggggtttcctcagtcagt

SEQ ID NO: 595 - DNA, 17 bp, synthetic construct
  source 1..17: mol_type = other DNA
cgtccctccgaatgtta

SEQ ID NO: 596 - DNA, 20 bp, synthetic construct
  source 1..20: mol_type = other DNA
cgttggctacccgtgatatt

SEQ ID NO: 597 - DNA, 22 bp, synthetic construct
  source 1..22: mol_type = other DNA
ctcgtcaagaaggcgatagaag

SEQ ID NO: 598 - DNA, 24 bp, synthetic construct
  source 1..24: mol_type = other DNA
ccgcttcctcgtgctttacggtat

SEQ ID NO: 599 - DNA, 20 bp, synthetic construct
  source 1..20: mol_type = other DNA
gggttccacgtccatcagta

SEQ ID NO: 600 - DNA, 20 bp, synthetic construct
  source 1..20: mol_type = other DNA
acaccgtcctttccagcagt

SEQ ID NO: 601 - DNA, 19 bp, synthetic construct
  source 1..19: mol_type = other DNA
tgcaccaccaactgcttag

SEQ ID NO: 602 - DNA, 19 bp, synthetic construct
  source 1..19: mol_type = other DNA
ggatgcagggatgatgttc

SEQ ID NO: 603 - DNA, 25 bp, synthetic construct
  source 1..25: mol_type = other DNA
cggcatcgctactcctctcatcaga

SEQ ID NO: 604 - DNA, 20 bp, synthetic construct
  source 1..20: mol_type = other DNA
gccacgatatggtctcctga

SEQ ID NO: 605 - DNA, 20 bp, synthetic construct
  source 1..20: mol_type = other DNA
gagcttctctgtgacccagt

SEQ ID NO: 606 - DNA, 21 bp, synthetic construct
  source 1..21: mol_type = other DNA
tctcggccttgactgtgccgt

SEQ ID NO: 607 - DNA, 20 bp, synthetic construct
  source 1..20: mol_type = other DNA
tatgactccactcacggcaa

SEQ ID NO: 608 - DNA, 20 bp, synthetic construct
  source 1..20: mol_type = other DNA
tggaagatggtgatgggctt

SEQ ID NO: 609 - DNA, 21 bp, synthetic construct
  source 1..21: mol_type = other DNA
tggcagagctgccttccgtct

SEQ ID NO: 610 - DNA, 20 bp, synthetic construct
  source 1..20: mol_type = other DNA
tggagtatggcttcacggtt

SEQ ID NO: 611 - DNA, 20 bp, synthetic construct
  source 1..20: mol_type = other DNA
tgcaggacttgggtgatctt

SEQ ID NO: 612 - DNA, 21 bp, synthetic construct
  source 1..21: mol_type = other DNA
tctcggccttgactgtgccgt

SEQ ID NO: 613 - DNA, 20 bp, synthetic construct
  source 1..20: mol_type = other DNA
tatgactccactcacggcaa

SEQ ID NO: 614 - DNA, 20 bp, synthetic construct
  source 1..20: mol_type = other DNA
tggaagatggtgatgggctt